European Patent Application EP 4 484 441 A1, published January 1, 2025. Title: MHC-class I derived polypeptide for targeting a capture molecule when bound to an oligopeptide. Applicant: Eberhard Karls Universität Tübingen Medizinische Fakultät. The sequence listing filed with the application follows.

SEQUENCE LISTING (10 sequences)

SEQ ID NO: 1 - protein, 30 aa, synthetic construct
SAWSHPQFEKGGGSGGGSGGSAWSHPQFEK

SEQ ID NO: 2 - protein, 6 aa, synthetic construct
GGGSGG

SEQ ID NO: 3 - protein, 15 aa, synthetic construct
GGGGSGGGGSGGGGS

SEQ ID NO: 4 - protein, 99 aa, synthetic construct [sequence omitted]

SEQ ID NO: 5 - protein, 426 aa, synthetic construct
IQRTPKIQVYSRHPAENGKSNFLNCYVSGFHPSDIEVDLLKNGERIEKVEHSDLSFSKDWSFYLLYYTEFTPTEKDEYACRVNHVTLSQPKIVKWDRDMGGGGSGGGGSGGGGSGSHSMRYFFTSVSRPGRGEPRFIAVGYVDDTQFVRFDSDAASQKMEPRAPWIEQEGPEYWDQETRNMKAHSQTDRANLGTLRGCYNQSEDGSHTIQIMYGCDVGPDGRFLRGYRQDAYDGKDYIALNEDLRSWTAADMCAQITKRKWEAVHAAEQRRVYLEGRCVDGLRRYLENGKETLQRTDPPKTHMTHHPISDHEATLRCWALGFYPAEITLTWQRDGEDQTQDTELVETRPAGDGTFQKWVAVVVPSGQEQRYTCHVQHEGLPKPLTLRWEPGGGSGGSAWSHPQFEKGGGSGGGSGGSAWSHPQFEK

SEQ ID NO: 6 - protein, 10 aa, synthetic construct
LTDLGQNLLY

SEQ ID NO: 7 - protein, 276 aa, synthetic construct
GSHSMRYFFTSVSRPGRGEPRFIAVGYVDDTQFVRFDSDAASQKMEPRAPWIEQEGPEYWDQETRNMKAHSQTDRANLGTLRGCYNQSEDGSHTIQIMYGCDVGPDGRFLRGYRQDAYDGKDYIALNEDLRSWTAADMCAQITKRKWEAVHAAEQRRVYLEGRCVDGLRRYLENGKETLQRTDPPKTHMTHHPISDHEATLRCWALGFYPAEITLTWQRDGEDQTQDTELVETRPAGDGTFQKWVAVVVPSGQEQRYTCHVQHEGLPKPLTLRWEP

SEQ ID NO: 8 - protein, 10 aa, synthetic construct
SAWSHPQFEK

SEQ ID NO: 9 - protein, 10 aa, synthetic construct
GGGSGGGSGG

SEQ ID NO: 10 - protein, 20 aa, synthetic construct
MSRSVALAVLALLSLSGLEA